European Patent Application EP 4 414 452 A1, published August 14, 2024. Title: DUAL-GUIDE RNA COMPOSITION FOR EXECUTING A SINGLE-GUIDE RNA CRISPR-ASSOCIATED SYSTEM. Applicant: UNIVERSIDAD DE GRANADA. The sequence listing filed with the application follows.

SEQUENCE LISTING (16 sequences)

SEQ ID NO: 1 - RNA, 42 nt, synthetic construct
  source 1..42: mol_type = other RNA
gatttagactaccccaaaaacgaaggggactaaaacgagcgc

SEQ ID NO: 2 - RNA, 44 nt, synthetic construct
  source 1..44: mol_type = other RNA
gatttagactaccccaaaaacgaaggggactaaaacgacagata

SEQ ID NO: 3 - RNA, 20 nt, synthetic construct
  source 1..20: mol_type = other RNA
taatttctactcttgtagat

SEQ ID NO: 4 - DNA, 85 bp, synthetic construct
  source 1..85: mol_type = other DNA
taaggcctgctgaaaatgactgaatataaacttgtggtagttggagctggtggcgtaggcaagagtgccttgacgatacagctaa

SEQ ID NO: 5 - DNA, 85 bp, synthetic construct
  source 1..85: mol_type = other DNA
taaggcctgctgaaaatgactgaatataaacttgtggtagttggagcttgtggcgtaggcaagagtgccttgacgatacagctaa

SEQ ID NO: 6 - DNA, 85 bp, synthetic construct
  source 1..85: mol_type = other DNA
taaggcctgctgaaaatgactgaatataaacttgtggtagttggagctgatggcgtaggcaagagtgccttgacgatacagctaa

SEQ ID NO: 7 - DNA, 85 bp, synthetic construct
  source 1..85: mol_type = other DNA
taaggcctgctgaaaatgactgaatataaacttgtggtagttggagctgttggcgtaggcaagagtgccttgacgatacagctaa

SEQ ID NO: 8 - RNA, 85 nt, synthetic construct
  source 1..85: mol_type = other RNA
taaggcctgctgaaaatgactgaatataaacttgtggtagttggagctggtggcgtaggcaagagtgccttgacgatacagctaa

SEQ ID NO: 9 - RNA, 85 nt, synthetic construct
  source 1..85: mol_type = other RNA
taaggcctgctgaaaatgactgaatataaacttgtggtagttggagcttgtggcgtaggcaagagtgccttgacgatacagctaa

SEQ ID NO: 10 - RNA, 85 nt, synthetic construct
  source 1..85: mol_type = other RNA
taaggcctgctgaaaatgactgaatataaacttgtggtagttggagctgatggcgtaggcaagagtgccttgacgatacagctaa

SEQ ID NO: 11 - RNA, 85 nt, synthetic construct
  source 1..85: mol_type = other RNA
taaggcctgctgaaaatgactgaatataaacttgtggtagttggagctgttggcgtaggcaagagtgccttgacgatacagctaa

SEQ ID NO: 12 - RNA, 64 nt, synthetic construct
  source 1..64: mol_type = other RNA
gatttagactaccccaaaaacgaaggggactaaaactgtaatggttccattttcattatatttt

SEQ ID NO: 13 - RNA, 42 nt, synthetic construct; identical to SEQ ID NO: 1
  source 1..42: mol_type = other RNA

SEQ ID NO: 14 - RNA, 33 nt, synthetic construct
  source 1..33: mol_type = other RNA
tcgcgttttatattacttttaccttggtaatgt

SEQ ID NO: 15 - RNA, 44 nt, synthetic construct; identical to SEQ ID NO: 2
  source 1..44: mol_type = other RNA

SEQ ID NO: 16 - RNA, 35 nt, synthetic construct
  source 1..35: mol_type = other RNA
tgtctatttttatattacttttaccttggtaatgt